European Patent Application EP 4 219 693 A1, published August 2, 2023. Title: Chimeric antigen receptor targeting CD7 and application thereof. Applicant: Bioheng Therapeutics Limited. The sequence listing filed with the application follows.

SEQUENCE LISTING (82 sequences)

SEQ ID NO: 1 - protein, 11 aa, Artificial Sequence
  CDR-L1
RASQSISNNLH

SEQ ID NO: 2 - protein, 7 aa, Artificial Sequence
  CDR-L2
SASQSIS

SEQ ID NO: 3 - protein, 9 aa, Artificial Sequence
  CDR-L3
QQSNSWPYT

SEQ ID NO: 4 - protein, 7 aa, Artificial Sequence
  CDR-H1
GYTFTSY

SEQ ID NO: 5 - protein, 6 aa, Artificial Sequence
  CDR-H2
NPSNGR

SEQ ID NO: 6 - protein, 14 aa, Artificial Sequence
  CDR-H3
GGVYYDLYYYALDY

SEQ ID NO: 7 - protein, 108 aa, Artificial Sequence
  m189 VL
DIELTQSPATLSVTPGDSVSLSCRASQSISNNLHWYQQKSHESPRLLIKSASQSISGIPSRFSGSGSGTDFTLSINSVETEDFGMYFCQQSNSWPYTFGGGTKLEIKR

SEQ ID NO: 8 - protein, 123 aa, Artificial Sequence
  m189 VH
QVQLQESGAELVKPGASVKLSCKASGYTFTSYWMHWVKQRPGQGLEWIGKINPSNGRTNYNEKFKSKATLTVDKSSSTAYMQLSSLTSEDSAVYYCARGGVYYDLYYYALDYWGQGTTVTVSS

SEQ ID NO: 9 - protein, 249 aa, Artificial Sequence
  m189 scFv
DIELTQSPATLSVTPGDSVSLSCRASQSISNNLHWYQQKSHESPRLLIKSASQSISGIPSRFSGSGSGTDFTLSINSVETEDFGMYFCQQSNSWPYTFGGGTKLEIKRGSTSGSGKPGSGEGSTKGQVQLQESGAELVKPGASVKLSCKASGYTFTSYWMHWVKQRPGQGLEWIGKINPSNGRTNYNEKFKSKATLTVDKSSSTAYMQLSSLTSEDSAVYYCARGGVYYDLYYYALDYWGQGTTVTVSS

SEQ ID NO: 10 - protein, 108 aa, Artificial Sequence
  h189-1 VL
EIVLTQSPATLSLSPGERATLSCRASQSISNNLHWYQQKPGQAPRLLIYSASQSISGIPARFSGSGPGTDFTLTISSLEPEDFAVYYCQQSNSWPYTFGQGTKVEIKR

SEQ ID NO: 11 - protein, 123 aa, Artificial Sequence
  h189-1 VH
QVQLVQSGAEVKKPGASVKVSCKASGYTFTSYYMHWVRQAPGQGLEWMGWINPSNGRTNYAQKFQGRVTMTRDTSISTAYMELSRLRSDDTAVYYCARGGVYYDLYYYALDYWGQGTLVTVSS

SEQ ID NO: 12 - protein, 249 aa, Artificial Sequence
  h189-1 scFv
EIVLTQSPATLSLSPGERATLSCRASQSISNNLHWYQQKPGQAPRLLIYSASQSISGIPARFSGSGPGTDFTLTISSLEPEDFAVYYCQQSNSWPYTFGQGTKVEIKRGSTSGSGKPGSGEGSTKGQVQLVQSGAEVKKPGASVKVSCKASGYTFTSYYMHWVRQAPGQGLEWMGWINPSNGRTNYAQKFQGRVTMTRDTSISTAYMELSRLRSDDTAVYYCARGGVYYDLYYYALDYWGQGTLVTVSS

SEQ ID NO: 13 - protein, 108 aa, Artificial Sequence
  h189-2 VL
DVVMTQSPAFLSVTPGEKVTITCRASQSISNNLHWYQQKPDQAPKLLIKSASQSISGVPSRFSGSGSGTDFTFTISSLEAEDAATYYCQQSNSWPYTFGQGTKVEIKR

SEQ ID NO: 14 - protein, 123 aa, Artificial Sequence; identical to SEQ ID NO: 11
  h189-2 VH

SEQ ID NO: 15 - protein, 249 aa, Artificial Sequence
  h189-2 scFv
DVVMTQSPAFLSVTPGEKVTITCRASQSISNNLHWYQQKPDQAPKLLIKSASQSISGVPSRFSGSGSGTDFTFTISSLEAEDAATYYCQQSNSWPYTFGQGTKVEIKRGSTSGSGKPGSGEGSTKGQVQLVQSGAEVKKPGASVKVSCKASGYTFTSYYMHWVRQAPGQGLEWMGWINPSNGRTNYAQKFQGRVTMTRDTSISTAYMELSRLRSDDTAVYYCARGGVYYDLYYYALDYWGQGTLVTVSS

SEQ ID NO: 16 - protein, 108 aa, Artificial Sequence
  h189-3 VL
DVVMTQSPAFLSVTPGEKVTITCRASQSISNNLHWYQQKPDQAPKLLIKSASQSISGVPSRFSGSGSGTDFTFTISSLEAEDAAMYFCQQSNSWPYTFGQGTKVEIKR

SEQ ID NO: 17 - protein, 123 aa, Artificial Sequence
  h189-3 VH
QVQLVQSGAEVKKPGASVKVSCKASGYTFTSYWMHWVRQAPGQGLEWMGKINPSNGRTNYAQKFQGRVTMTRDTSISTAYMELSRLRSDDTAVYYCARGGVYYDLYYYALDYWGQGTLVTVSS

SEQ ID NO: 18 - protein, 249 aa, Artificial Sequence
  h189-3 scFv
DVVMTQSPAFLSVTPGEKVTITCRASQSISNNLHWYQQKPDQAPKLLIKSASQSISGVPSRFSGSGSGTDFTFTISSLEAEDAAMYFCQQSNSWPYTFGQGTKVEIKRGSTSGSGKPGSGEGSTKGQVQLVQSGAEVKKPGASVKVSCKASGYTFTSYWMHWVRQAPGQGLEWMGKINPSNGRTNYAQKFQGRVTMTRDTSISTAYMELSRLRSDDTAVYYCARGGVYYDLYYYALDYWGQGTLVTVSS

SEQ ID NO: 19 - protein, 108 aa, Artificial Sequence
  h189-4 VL
EIVLTQSPATLSLSPGERATLSCRASQSISNNLHWYQQKPGQAPRLLIKSASQSISGIPARFSGSGPGTDFTLTISSLEPEDFAVYFCQQSNSWPYTFGQGTKVEIKR

SEQ ID NO: 20 - protein, 123 aa, Artificial Sequence; identical to SEQ ID NO: 17
  h189-4 VH

SEQ ID NO: 21 - protein, 249 aa, Artificial Sequence
  h189-4 scFv
EIVLTQSPATLSLSPGERATLSCRASQSISNNLHWYQQKPGQAPRLLIKSASQSISGIPARFSGSGPGTDFTLTISSLEPEDFAVYFCQQSNSWPYTFGQGTKVEIKRGSTSGSGKPGSGEGSTKGQVQLVQSGAEVKKPGASVKVSCKASGYTFTSYWMHWVRQAPGQGLEWMGKINPSNGRTNYAQKFQGRVTMTRDTSISTAYMELSRLRSDDTAVYYCARGGVYYDLYYYALDYWGQGTLVTVSS

SEQ ID NO: 22 - protein, 25 aa, Artificial Sequence
  CD8alpha transmembrane domain
IYIWAPLAGTCGVLLLSLVITLYCK

SEQ ID NO: 23 - DNA, 75 bp, Artificial Sequence
  CD8alpha transmembrane domain
atctacatctgggcgcccttggccgggacttgtggggtccttctcctgtcactggttatcaccctttactgcaaa

SEQ ID NO: 24 - protein, 27 aa, Artificial Sequence
  CD28 transmembrane domain
FWVLVVVGGVLACYSLLVTVAFIIFWV

SEQ ID NO: 25 - DNA, 81 bp, Artificial Sequence
  CD28 transmembrane domain
ttttgggtcctcgtcgtagttggaggggtacttgcctgttatagcctcctggttaccgtagcatttattatattctgggtg

SEQ ID NO: 26 - protein, 41 aa, Artificial Sequence
  CD28 costimulatory domain
RSKRSRLLHSDYMNMTPRRPGPTRKHYQPYAPPRDFAAYRS

SEQ ID NO: 27 - DNA, 123 bp, Artificial Sequence
  CD28 costimulatory domain
aggagtaagaggagcaggctcctgcacagtgactacatgaacatgactccccgccgccccgggcccacccgcaagcattaccagccctatgccccaccacgcgacttcgcagcctatcgctcc

SEQ ID NO: 28 - protein, 40 aa, Artificial Sequence
  4-1BB costimulatory domain
RGRKKLLYIFKQPFMRPVQTTQEEDGCSCRFPEEEEGGCE

SEQ ID NO: 29 - DNA, 120 bp, Artificial Sequence
  4-1BB costimulatory domain
cggggcagaaagaaactcctgtatatattcaaacaaccatttatgagaccagtacaaactactcaagaggaagatggctgtagctgccgatttccagaagaagaagaaggaggatgtgaa

SEQ ID NO: 30 - protein, 113 aa, Artificial Sequence
  CD3zeta signaling domain
LRVKFSRSADAPAYQQGQNQLYNELNLGRREEYDVLDKRRGRDPEMGGKPRRKNPQEGLYNELQKDKMAEAYSEIGMKGERRRGKGHDGLYQGLSTATKDTYDALHMQALPPR

SEQ ID NO: 31 - DNA, 339 bp, Artificial Sequence
  CD3zeta signaling domain
ctgagagtgaagttcagcaggagcgcagacgcccccgcgtaccagcagggccagaaccagctctataacgagctcaatctaggacgaagagaggagtacgatgttttggacaagagacgtggccgggaccctgagatggggggaaagccgagaaggaagaaccctcaggaaggcctgtacaatgaactgcagaaagataagatggcggaggcctacagtgagattgggatgaaaggcgagcgccggaggggcaaggggcacgatggcctttaccagggtctcagtacagccaccaaggacacctacgacgcccttcacatgcaggccctgccccctcgc

SEQ ID NO: 32 - protein, 114 aa, Artificial Sequence
  CD3zeta signaling domain
LRVKFSRSADAPAYQQGQNQLFNELNLGRREEFDVLDKRRGRDPEMGGKPQRRKNPQEGLYNELQKDKMAEAYSEIGMKGERRRGKGHDGLFQGLSTATKDTFDALHMQALPPR

SEQ ID NO: 33 - DNA, 342 bp, Artificial Sequence
  CD3zeta signaling domain
ctgagagtgaagttcagcaggagcgcagacgcccccgcgtaccagcagggccagaaccagctctttaacgagctcaatctaggacgaagagaggagttcgatgttttggacaagagacgtggccgggaccctgagatggggggaaagccgcagagaaggaagaaccctcaggaaggcctgtacaatgaactgcagaaagataagatggcggaggcctacagtgagattgggatgaaaggcgagcgccggaggggcaaggggcacgatggccttttccagggtctcagtacagccaccaaggacacctttgacgcccttcacatgcaggccctgccccctcgc

SEQ ID NO: 34 - protein, 20 aa, Artificial Sequence
  B2M signal peptide
MSRSVALAVLALLSLSGLEA

SEQ ID NO: 35 - DNA, 60 bp, Artificial Sequence
  B2M signal peptide
atgtcccgctctgttgctttggctgtgctggcccttttgtcccttagcggactggaggcc

SEQ ID NO: 36 - protein, 21 aa, Artificial Sequence
  CD8alpha signal peptide
MALPVTALLLPLALLLHAARP

SEQ ID NO: 37 - DNA, 63 bp, Artificial Sequence
  CD8alpha signal peptide
atggccttaccagtgaccgccttgctcctgccgctggccttgctgctccacgccgccaggccg

SEQ ID NO: 38 - protein, 45 aa, Artificial Sequence
  CD8alpha hinge region
TTTPAPRPPTPAPTIASQPLSLRPEACRPAAGGAVHTRGLDFACD

SEQ ID NO: 39 - DNA, 135 bp, Artificial Sequence
  CD8alpha hinge region
accacgacgccagcgccgcgaccaccaacaccggcgcccaccatcgcgtcgcagcccctgtccctgcgcccagaggcgtgccggccagcggcggggggcgcagtgcacacgagggggctggacttcgcctgtgat

SEQ ID NO: 40 - protein, 39 aa, Artificial Sequence
  CD28 hinge region
IEVMYPPPYLDNEKSNGTIIHVKGKHLCPSPLFPGPSKP

SEQ ID NO: 41 - DNA, 117 bp, Artificial Sequence
  CD28 hinge region
attgaagttatgtatcctcctccttacctagacaatgagaagagcaatggaaccattatccatgtgaaagggaaacacctttgtccaagtcccctatttcccggaccttctaagccc

SEQ ID NO: 42 - protein, 12 aa, Artificial Sequence
  IgG4 hinge region
ESKYGPPCPPCP

SEQ ID NO: 43 - DNA, 36 bp, Artificial Sequence
  IgG4 hinge region
gaaagcaaatacgggccgccgtgtccaccctgtccg

SEQ ID NO: 44 - protein, 18 aa, Artificial Sequence
  PD-L1 signal peptide
MRIFAVFIFMTYWHLLNA

SEQ ID NO: 45 - protein, 223 aa, Artificial sequence
  PDL1 extracellular domain
FTVTVPKDLYVVEYGSNMTIECKFPVEKQLDLAALIVYWEMEDKNIIQFVHGEEDLKVQHSSYRQRARLLKDQLSLGNAALQITDVKLQDAGVYRCMISYGGADYKRITVKVNAPYNKINQRILVVDPVTSEHELTCQAEGYPKAEVIWTSSDHQVLSGKTTTTNSKREEKLFNVTSTLRINTTTNEIFYCTFRRLDPEENHTAELVIPELPLAHPPNERTHL

SEQ ID NO: 46 - protein, 201 aa, Artificial sequence
  PDL2 extracellular domain
LFTVTVPKELYIIEHGSNVTLECNFDTGSHVNLGAITASLQKVENDTSPHRERATLLEEQLPLGKASFHIPQVQVRDEGQYQCIIIYGVAWDYKYLTLKVKASYRKINTHILKVPETDEVELTCQATGYPLAEVSWPNVSVPANTSHSRTPEGLYQVTSVLRLKPPPGRNFSCVFWNTHVRELTLASIDLQSQMEPRTHPT

SEQ ID NO: 47 - protein, 356 aa, Artificial sequence
  E- cadherin EC1-EC2
WLCQEPEPCHPGFDAESYTFTVPRRHLERGRVLGRVNFEDCTGRQRTAYFSLDTRFKVGTDGVITVKRPLRFHNPQIHFLVYAWDSTYRKFSTKVTLNTVGHHHRPPPHQASVSGIQAELLTFPNSSPGLRRQKRDWVIPPISCPENEKGPFPKNLVQIKSNKDKEGKVFYSITGQGADTPPVGVFIIERETGWLKVTEPLDRERIATYTLFSHAVSSNGNAVEDPMEILITVTDQNDNKPEFTQEVFKGSVMEGALPGTSVMEVTATDADDDVNTYNAAIAYTILSQDPELPDKNMFTINRNTGVISVVTTGLDRESFPTYTLVVQAADLQGEGLSTTATAVITVTDTNDNPPIF

SEQ ID NO: 48 - protein, 689 aa, Artificial sequence
  E- cadherin EC1-EC5
WLCQEPEPCHPGFDAESYTFTVPRRHLERGRVLGRVNFEDCTGRQRTAYFSLDTRFKVGTDGVITVKRPLRFHNPQIHFLVYAWDSTYRKFSTKVTLNTVGHHHRPPPHQASVSGIQAELLTFPNSSPGLRRQKRDWVIPPISCPENEKGPFPKNLVQIKSNKDKEGKVFYSITGQGADTPPVGVFIIERETGWLKVTEPLDRERIATYTLFSHAVSSNGNAVEDPMEILITVTDQNDNKPEFTQEVFKGSVMEGALPGTSVMEVTATDADDDVNTYNAAIAYTILSQDPELPDKNMFTINRNTGVISVVTTGLDRESFPTYTLVVQAADLQGEGLSTTATAVITVTDTNDNPPIFNPTTYKGQVPENEANVVITTLKVTDADAPNTPAWEAVYTILNDDGGQFVVTTNPVNNDGILKTAKGLDFEAKQQYILHVAVTNVVPFEVSLTTSTATVTVDVLDVNEAPIFVPPEKRVEVSEDFGVGQEITSYTAQEPDTFMEQKITYRIWRDTANWLEINPDTGAISTRAELDREDFEHVKNSTYTALIIATDNGSPVATGTGTLLLILSDVNDNAPIPEPRTIFFCERNPKPQVINIIDADLPPNTSPFTAELTHGASANWTIQYNDPTQESIILKPKMALEVGDYKINLKLMDNQNKDQVTTLEVSVCDCEGAAGVCRKAQPVEAGLQIP

SEQ ID NO: 49 - protein, 283 aa, Artificial sequence
  HLA-G extracellular domain
GSHSMRYFSAAVSRPGRGEPRFIAMGYVDDTQFVRFDSDSACPRMEPRAPWVEQEGPEYWEEETRNTKAHAQTDRMNLQTLRGYYNQSEASSHTLQWMIGCDLGSDGRLLRGYEQYAYDGKDYLALNEDLRSWTAADTAAQISKRKCEAANVAEQRRAYLEGTCVEWLHRYLENGKEMLQRADPPKTHVTHHPVFDYEATLRCWALGFYPAEIILTWQRDGEDQTQDVELVETRPAGDGTFQKWAAVVVPSGEEQRYTCHVQHEGLPEPLMLRWKQSSLPTIP

SEQ ID NO: 50 - protein, 284 aa, Artificial Sequence
  HLA-E extracellular domain
GSHSLKYFHTSVSRPGRGEPRFISVGYVDDTQFVRFDNDAASPRMVPRAPWMEQEGSEYWDRETRSARDTAQIFRVNLRTLRGYYNQSEAGSHTLQWMHGCELGPDGRFLRGYEQFAYDGKDYLTLNEDLRSWTAVDTAAQISEQKSNDASEAEHQRAYLEDTCVEWLHKYLEKGKETLLHLEPPKTHVTHHPISDHEATLRCWALGFYPAEITLTWQQDGEGHTQDTELVETRPAGDGTFQKWAAVVVPSGEEQRYTCHVQHEGLPEPVTLRWKPASQPTIPI

SEQ ID NO: 51 - protein, 284 aa, Artificial Sequence
  HLA-G extracellular domain mutant
GSHSLKYFHTSVSRPGRGEPRFISVGYVDDTQFVRFDNDAASPRMVPRAPWMEQEGSEYWDRETRSARDTAQIFRVNLRTLRGCYNQSEAGSHTLQWMHGCELGPDGRFLRGYEQFAYDGKDYLTLNEDLRSWTAVDTAAQISEQKSNDASEAEHQRAYLEDTCVEWLHKYLEKGKETLLHLEPPKTHVTHHPISDHEATLRCWALGFYPAEITLTWQQDGEGHTQDTELVETRPAGDGTFQKWAAVVVPSGEEQRYTCHVQHEGLPEPVTLRWKPASQPTIPI

SEQ ID NO: 52 - protein, 107 aa, Artificial Sequence
  CD19 scFv-1 VL
DIQMTQTTSSLSASLGDRVTISCRASQDISKYLNWYQQKPDGTVKLLIYHTSRLHSGVPSRFSGSGSGTDYSLTISNLEQEDIATYFCQQGNTLPYTFGGGTKLEIT

SEQ ID NO: 53 - protein, 120 aa, Artificial Sequence
  CD19 scFv-1 VH
EVKLQESGPGLVAPSQSLSVTCTVSGVSLPDYGVSWIRQPPRKGLEWLGVIWGSETTYYNSALKSRLTIIKDNSKSQVFLKMNSLQTDDTAIYYCACHYYYGGSYAMDYWGQGTSVTVSS

SEQ ID NO: 54 - protein, 242 aa, Artificial Sequence
  CD19 scFv-1
DIQMTQTTSSLSASLGDRVTISCRASQDISKYLNWYQQKPDGTVKLLIYHTSRLHSGVPSRFSGSGSGTDYSLTISNLEQEDIATYFCQQGNTLPYTFGGGTKLEITGGGGSGGGGSGGGGSEVKLQESGPGLVAPSQSLSVTCTVSGVSLPDYGVSWIRQPPRKGLEWLGVIWGSETTYYNSALKSRLTIIKDNSKSQVFLKMNSLQTDDTAIYYCAKHYYYGGSYAMDYWGQGTSVTVSS

SEQ ID NO: 55 - protein, 107 aa, Artificial Sequence
  CD19 scFv-2 VL
DIQMTQSPASLSTSLGETVTIQCQASEDIYSGLAWYQQKPGKSPQLLIYGASDLQDGVPSRFSGSGSGTQYSLKITSMQTEDEGVYFCQQGLTYPRTFGGGTKLELK

SEQ ID NO: 56 - protein, 116 aa, Artificial Sequence
  CD19 scFv-2 VH
EVQLQQSGAELVRPGTSVKLSCKVSGDTITFYYMHFVKQRPGQGLEWIGRIDPEDESTKYSEKFKNKATLTADTSSNTAYLKLSSLTSEDTATYFCIYGGYYFDYWGQGVMVTVSS

SEQ ID NO: 57 - protein, 238 aa, Artificial Sequence
  CD19 scFv-2
DIQMTQSPASLSTSLGETVTIQCQASEDIYSGLAWYQQKPGKSPQLLIYGASDLQDGVPSRFSGSGSGTQYSLKITSMQTEDEGVYFCQQGLTYPRTFGGGTKLELKGGGGSGGGGSGGGGSEVQLQQSGAELVRPGTSVKLSCKVSGDTITFYYMHFVKQRPGQGLEWIGRIDPEDESTKYSEKFKNKATLTADTSSNTAYLKLSSLTSEDTATYFCIYGGYYFDYWGQGVMVTVSS

SEQ ID NO: 58 - protein, 119 aa, Artificial sequence
  mNKG2A scFv-VH
EVQLVESGGGLVKPGGSLKLSCAASGFTFSSYAMSWVRQSPEKRLEWVAEISSGGSYTYYPDTVTGRFTISRDNAKNTLYLEISSLRSEDTAMYYCTRHGDYPRFFDVWGAGTTVTVSS

SEQ ID NO: 59 - protein, 107 aa, Artificial sequence
  mNKG2A scFv-VL
QIVLTQSPALMSASPGEKVTMTCSASSSVSYIYWYQQKPRSSPKPWIYLTSNLASGVPARFSGSGSGTSYSLTISSMEAEDAATYYCQQWSGNPYTFGGGTKLEIKR

SEQ ID NO: 60 - protein, 244 aa, Artificial sequence
  mNKG2A scFv
QIVLTQSPALMSASPGEKVTMTCSASSSVSYIYWYQQKPRSSPKPWIYLTSNLASGVPARFSGSGSGTSYSLTISSMEAEDAATYYCQQWSGNPYTFGGGTKLEIKRGSTSGSGKPGSGEGSTKGEVQLVESGGGLVKPGGSLKLSCAASGFTFSSYAMSWVRQSPEKRLEWVAEISSGGSYTYYPDTVTGRFTISRDNAKNTLYLEISSLRSEDTAMYYCTRHGDYPRFFDVWGAGTTVTVSS

SEQ ID NO: 61 - protein, 119 aa, Artificial sequence
  hNKG2A scFv-VH
EVQLVESGGGLVKPGGSLRLSCAASGFTFSSYAKSWVRQAPGKGLEWVSEISSGGSYTYYADSVKGRFTISRDNAKNSLYLQMNSLRAEDTAVYYCARHGDYPRFFDVWGQGTTVTVSS

SEQ ID NO: 62 - protein, 107 aa, Artificial sequence
  hNKG2A scFv-VL
EIVLTQSPATLSLSPGERATLSCSASSSVSSYIYWYQQKPGQAPRLLIYLTSNLASGIPARFSGSGSGTDFTLTISSLEPEDFAVYYCQQWSGNPYTFGQGTKLEIK

SEQ ID NO: 63 - protein, 244 aa, Artificial sequence
  hNKG2A scFv
EIVLTQSPATLSLSPGERATLSCSASSSVSSYIYWYQQKPGQAPRLLIYLTSNLASGIPARFSGSGSGTDFTLTISSLEPEDFAVYYCQQWSGNPYTFGQGTKLEIKGSTSGSGKPGSGEGSTKGEVQLVESGGGLVKPGGSLRLSCAASGFTFSSYAKSWVRQAPGKGLEWVSEISSGGSYTYYADSVKGRFTISRDNAKNSLYLQMNSLRAEDTAVYYCARHGDYPRFFDVWGQGTTVTVSS

SEQ ID NO: 64 - protein, 15 aa, Artificial sequence
  linker
GGGGSGGGGSGGGGS

SEQ ID NO: 65 - protein, 108 aa, Artificial sequence
  KIR scFv VL
EIVLTQSPVTLSLSPGERATLSCRASQSVSSYLAWYQQKPGQAPRLLIYDASNRATGIPARFSGSGSGTDFTLTISSLEPEDFAVYYCQQRSNWMYTFGQGTKLEIKR

SEQ ID NO: 66 - protein, 123 aa, Artificial sequence
  KIR scFv VH
QVQLVQSGAEVKKPGSSVKVSCKASGGTFSFYAISWVRQAPGQGLEWMGGFIPIFGAANYAQKFQGRVTITADESTSTAYMELSSLRSDDTAVYYCARIPSGSYYYDYDMDVWGQGTTVTVSS

SEQ ID NO: 67 - protein, 246 aa, Artificial sequence
  KIR scFv
QVQLVQSGAEVKKPGSSVKVSCKASGGTFSFYAISWVRQAPGQGLEWMGGFIPIFGAANYAQKFQGRVTITADESTSTAYMELSSLRSDDTAVYYCARIPSGSYYYDYDMDVWGQGTTVTVSSGGGGSGGGGSGGGGSEIVLTQSPVTLSLSPGERATLSCRASQSVSSYLAWYQQKPGQAPRLLIYDASNRATGIPARFSGSGSGTDFTLTISSLEPEDFAVYYCQQRSNWMYTFGQGTKLEIKR

SEQ ID NO: 68 - protein, 107 aa, Artificial sequence
  LIR1 scFv-1 VL
DILLTQSPAILSVSPGERVSFSCRASQSIGTNIHWYQQRTNGSPRLLIKYASESISGIPSRFSGSGSGTDFTLTINSVESEDIADYYCQQSYSWPYTFGGGTKLEIK

SEQ ID NO: 69 - protein, 118 aa, Artificial sequence
  LIR1 scFv-1 VH
QVTLKESGPGILKPSQTLSLTCSFSGFSLSTSGLGVGWIRQPSGKGLEWLAHIWWDDDKYYLPSLKSQLTISKDTSRNQVFLKITSVDTADTATYYCARTELGRGDYWGQGTSVAVSS

SEQ ID NO: 70 - protein, 243 aa, Artificial sequence
  LIR1 scFv-2
DILLTQSPAILSVSPGERVSFSCRASQSIGTNIHWYQQRTNGSPRLLIKYASESISGIPSRFSGSGSGTDFTLTINSVESEDIADYYCQQSYSWPYTFGGGTKLEIKGSTSGSGKPGSGEGSTKGQVTLKESGPGILKPSQTLSLTCSFSGFSLSTSGLGVGWIRQPSGKGLEWLAHIWWDDDKYYLPSLKSQLTISKDTSRNQVFLKITSVDTADTATYYCARTELGRGDYWGQGTSVAVSS

SEQ ID NO: 71 - protein, 121 aa, Artificial sequence
  LIR1 scFv-2 VL
EVQLQQSGTVLPRPGASVKMSCKASGYSFTNYWMHWVKQRPGQGLEWIGAIYPGNSDTSYNQKFEGKAKLTAVTSASTAYMELSSLTNEDSAVYYCTTYDGYYSAWFAYWGQGTLVTVSAA

SEQ ID NO: 72 - protein, 108 aa, Artificial sequence
  LIR1 scFv-2 VH
DIVMTQSHKFMSTSVGDRVSITCKASQDVSTAVAWYQQKPGQSPKLLIYSASYRYTGVPDRFTGSGSGTDFTFTISSVQAEDLALYYCQQHYSPPWTFGGGTKLEIKR

SEQ ID NO: 73 - protein, 244 aa, Artificial sequence
  LIR1 scFv-2
EVQLQQSGTVLPRPGASVKMSCKASGYSFTNYWMHWVKQRPGQGLEWIGAIYPGNSDTSYNQKFEGKAKLTAVTSASTAYMELSSLTNEDSAVYYCTTYDGYYSAWFAYWGQGTLVTVSAAGGGGSGGGGSGGGGSDIVMTQSHKFMSTSVGDRVSITCKASQDVSTAVAWYQQKPGQSPKLLIYSASYRYTGVPDRFTGSGSGTDFTFTISSVQAEDLALYYCQQHYSPPWTFGGGTKLEIKR

SEQ ID NO: 74 - protein, 99 aa, Artificial sequence [sequence omitted]

SEQ ID NO: 75 - protein, 9 aa, Artificial sequence
  presenting peptide
VMAPRTLIL

SEQ ID NO: 76 - protein, 124 aa, Artificial sequence
  NKG2A scFv VH
QVQLVQSGAEVKKPGASVKVSCKASGYTFTSYWMNWVRQAPGQGLEWMGRIDPYDSETHYAQKLQGRVTMTTDTSTSTAYMELRSLRSDDTAVYYCARGGYDFDVGTLYWFFDVWGQGTTVTVS

SEQ ID NO: 77 - protein, 107 aa, Artificial sequence
  NKG2A scFv VL
DIQMTQSPSSLSASVGDRVTITCRASENIYSYLAWYQQKPGKAPKLLIYNAKTLAEGVPSRFSGSGSGTDFTLTISSLQPEDFATYYCQHHYGTPRTFGGGTKVEIK

SEQ ID NO: 78 - protein, 246 aa, Artificial sequence
  NKG2A scFv
DIQMTQSPSSLSASVGDRVTITCRASENIYSYLAWYQQKPGKAPKLLIYNAKTLAEGVPSRFSGSGSGTDFTLTISSLQPEDFATYYCQHHYGTPRTFGGGTKVEIKGGGGSGGGGSGGGGSQVQLVQSGAEVKKPGASVKVSCKASGYTFTSYWMNWVRQAPGQGLEWMGRIDPYDSETHYAQKLQGRVTMTTDTSTSTAYMELRSLRSDDTAVYYCARGGYDFDVGTLYWFFDVWGQGTTVTVS

SEQ ID NO: 79 - protein, 109 aa, Artificial sequence
  KIR scFv VL
EIVLTQSPVTLSLSPGERATLSCRASQSVSSYLAWYQQKPGQAPRLLIYDASNRATGIPARFSGSGSGTDFTLTISSLEPEDFAVYYCQQRSNWMYTFGQGTKLEIKRT

SEQ ID NO: 80 - protein, 123 aa, Artificial sequence; identical to SEQ ID NO: 66
  KIR scFv VH

SEQ ID NO: 81 - protein, 247 aa, Artificial sequence
  KIR scFv
EIVLTQSPVTLSLSPGERATLSCRASQSVSSYLAWYQQKPGQAPRLLIYDASNRATGIPARFSGSGSGTDFTLTISSLEPEDFAVYYCQQRSNWMYTFGQGTKLEIKRTGGGGSGGGGSGGGGSQVQLVQSGAEVKKPGSSVKVSCKASGGTFSFYAISWVRQAPGQGLEWMGGFIPIFGAANYAQKFQGRVTITADESTSTAYMELSSLRSDDTAVYYCARIPSGSYYYDYDMDVWGQGTTVTVSS

SEQ ID NO: 82 - DNA, 297 bp, Artificial sequence
  B2M with synonymous mutation
atccagaggaccccgaagatccaggtttattctcggcatcctgccgaaaatggaaaaagcaattttctcaactgttatgtgtctggatttcacccatctgacatagaggttgaccttcttaagaatggcgagagaatcgagaaggtcgaacattcagacttgagcttcagcaaggattggagcttttatcttctttattatactgaatttactcccactgaaaaggatgaatacgcctgcagggtaaaccatgtaacactcagtcagccaaagatcgtaaaatgggaccgagacatg